European Patent Application EP 4 317 182 A1, published February 7, 2024. Title: ANTIGEN-BINDING PROTEIN TARGETING STREPTOCOCCUS PNEUMONIAE HEMOLYSIN AND USE THEREOF. Applicant: STARMAB BIOLOGICS (SUZHOU) CO., LTD STARMAB BIOLOGICS (SHANGHAI) CO., LTD. The sequence listing filed with the application follows.

SEQUENCE LISTING (46 sequences)

SEQ ID NO: 1 - protein, 15 aa, Artificial Sequence
  HCDR3
TRTQFITSVVAPFDF

SEQ ID NO: 2 - protein, 10 aa, Artificial Sequence
  HCDR2
IRLKSNNYAT

SEQ ID NO: 3 - protein, 8 aa, Artificial Sequence
  HCDR1
GYTFGDNW

SEQ ID NO: 4 - protein, 9 aa, Artificial Sequence
  LCDR3
QQYYRYPLT

SEQ ID NO: 5 - protein, 2 aa, Artificial Sequence
  LCDR2
WA

SEQ ID NO: 6 - protein, 12 aa, Artificial Sequence
  LCDR1
QSLLYSRNQKNY

SEQ ID NO: 7 - protein, 25 aa, Artificial Sequence
  m2E5 H-FR1
EVKVEESGGGSVQPGGSMKLSCVAS

SEQ ID NO: 8 - protein, 17 aa, Artificial Sequence
  m2E5 H-FR2
MNWVRQSPEKGLEWVAE

SEQ ID NO: 9 - protein, 38 aa, Artificial Sequence
  m2E5 H-FR3
RYAESVKGRFTISRDDSKSSVYLQMNNLRTEDTGIYYC

SEQ ID NO: 10 - protein, 11 aa, Artificial Sequence
  m2E5 H-FR4
WGQGTTLTVSS

SEQ ID NO: 11 - protein, 26 aa, Artificial Sequence
  m2E5 L-FR1
DIVMSQSPSSLGVSVGEKITMSCKSS

SEQ ID NO: 12 - protein, 17 aa, Artificial Sequence
  m2E5 L-FR2
LAWYQQKPGQSPKLLIY

SEQ ID NO: 13 - protein, 37 aa, Artificial Sequence
  m2E5 L-FR3
STRESGVPDRFTGSGSGTDFTLTISSVKAEDLAVYYC

SEQ ID NO: 14 - protein, 10 aa, Artificial Sequence
  m2E5 L-FR4hu2E5 L-FR4
FGGGTKVEIK

SEQ ID NO: 15 - protein, 25 aa, Artificial Sequence
  hu2E5 H-FR1
EVQLVESGGGLVQPGGSLKLSCAAS

SEQ ID NO: 16 - protein, 17 aa, Artificial Sequence
  hu2E5 H-FR2
MNWVRQASGKGLEWVGE

SEQ ID NO: 17 - protein, 38 aa, Artificial Sequence
  hu2E5 H-FR3
RYAESVKGRFTISRDDSKNTVYLQMNSLKTEDTAVYYC

SEQ ID NO: 18 - protein, 11 aa, Artificial Sequence
  hu2E5 H-FR4
WGQGTTVTVSS

SEQ ID NO: 19 - protein, 26 aa, Artificial Sequence
  hu2E5 L-FR1
DIVMTQSPDSLAVSLGERATINCKSS

SEQ ID NO: 20 - protein, 17 aa, Artificial Sequence
  hu2E5 L-FR2
LAWYQQKPGQPPKLLIY

SEQ ID NO: 21 - protein, 37 aa, Artificial Sequence
  hu2E5 L-FR3
STRESGVPDRFSGSGSGTDFTLTISSLQAEDVAVYYC

SEQ ID NO: 22 - protein, 124 aa, Artificial Sequence
  m2E5 VH
EVKVEESGGGSVQPGGSMKLSCVASGYTFGDNWMNWVRQSPEKGLEWVAEIRLKSNNYATRYAESVKGRFTISRDDSKSSVYLQMNNLRTEDTGIYYCTRTQFITSVVAPFDFWGQGTTLTVSS

SEQ ID NO: 23 - protein, 113 aa, Artificial Sequence
  m2E5 VL
DIVMSQSPSSLGVSVGEKITMSCKSSQSLLYSRNQKNYLAWYQQKPGQSPKLLIYWASTRESGVPDRFTGSGSGTDFTLTISSVKAEDLAVYYCQQYYRYPLTFGGGTKVEIK

SEQ ID NO: 24 - protein, 124 aa, Artificial Sequence
  hu2E5 VH3
EVQLVESGGGLVQPGGSLKLSCAASGYTFGDNWMNWVRQASGKGLEWVGEIRLKSNNYATRYAESVKGRFTISRDDSKNTVYLQMNSLKTEDTAVYYCTRTQFITSVVAPFDFWGQGTTVTVSS

SEQ ID NO: 25 - protein, 113 aa, Artificial Sequence
  hu2E5VL0
DIVMTQSPDSLAVSLGERATINCKSSQSLLYSRNQKNYLAWYQQKPGQPPKLLIYWASTRESGVPDRFSGSGSGTDFTLTISSLQAEDVAVYYCQQYYRYPLTFGGGTKVEIK

SEQ ID NO: 26 - protein, 330 aa, Artificial Sequence
  IgG1
ASTKGPSVFPLAPSSKSTSGGTAALGCLVKDYFPEPVTVSWNSGALTSGVHTFPAVLQSSGLYSLSSVVTVPSSSLGTQTYICNVNHKPSNTKVDKRVEPKSCDKTHTCPPCPAPELLGGPSVFLFPPKPKDTLYITREPEVTCVVVDVSHEDPEVKFNWYVDGVEVHNAKTKPREEQYNSTYRVVSVLTVLHQDWLNGKEYKCKVSNKALPAPIEKTISKAKGQPREPQVYTLPPSREEMTKNQVSLTCLVKGFYPSDIAVEWESNGQPENNYKTTPPVLDSDGSFFLYSKLTVDKSRWQQGNVFSCSVMHEALHNHYTQKSLSLSPGK

SEQ ID NO: 27 - protein, 107 aa, Artificial Sequence [sequence omitted]

SEQ ID NO: 28 - protein, 454 aa, Artificial Sequence
  c2E5VHCH
EVKVEESGGGSVQPGGSMKLSCVASGYTFGDNWMNWVRQSPEKGLEWVAEIRLKSNNYATRYAESVKGRFTISRDDSKSSVYLQMNNLRTEDTGIYYCTRTQFITSVVAPFDFWGQGTTLTVSSASTKGPSVFPLAPSSKSTSGGTAALGCLVKDYFPEPVTVSWNSGALTSGVHTFPAVLQSSGLYSLSSVVTVPSSSLGTQTYICNVNHKPSNTKVDKRVEPKSCDKTHTCPPCPAPELLGGPSVFLFPPKPKDTLYITREPEVTCVVVDVSHEDPEVKFNWYVDGVEVHNAKTKPREEQYNSTYRVVSVLTVLHQDWLNGKEYKCKVSNKALPAPIEKTISKAKGQPREPQVYTLPPSREEMTKNQVSLTCLVKGFYPSDIAVEWESNGQPENNYKTTPPVLDSDGSFFLYSKLTVDKSRWQQGNVFSCSVMHEALHNHYTQKSLSLSPGK

SEQ ID NO: 29 - protein, 220 aa, Artificial Sequence
  c2E5VLCL
DIVMSQSPSSLGVSVGEKITMSCKSSQSLLYSRNQKNYLAWYQQKPGQSPKLLIYWASTRESGVPDRFTGSGSGTDFTLTISSVKAEDLAVYYCQQYYRYPLTFGGGTKVEIKRTVAAPSVFIFPPSDEQLKSGTASVVCLLNNFYPREAKVQWKVDNALQSGNSQESVTEQDSKDSTYSLSSTLTLSKADYEKHKVYACEVTHQGLSSPVTKSFNRGEC

SEQ ID NO: 30 - protein, 454 aa, Artificial Sequence
  hu2E5VH3CH
EVQLVESGGGLVQPGGSLKLSCAASGYTFGDNWMNWVRQASGKGLEWVGEIRLKSNNYATRYAESVKGRFTISRDDSKNTVYLQMNSLKTEDTAVYYCTRTQFITSVVAPFDFWGQGTTVTVSSASTKGPSVFPLAPSSKSTSGGTAALGCLVKDYFPEPVTVSWNSGALTSGVHTFPAVLQSSGLYSLSSVVTVPSSSLGTQTYICNVNHKPSNTKVDKRVEPKSCDKTHTCPPCPAPELLGGPSVFLFPPKPKDTLYITREPEVTCVVVDVSHEDPEVKFNWYVDGVEVHNAKTKPREEQYNSTYRVVSVLTVLHQDWLNGKEYKCKVSNKALPAPIEKTISKAKGQPREPQVYTLPPSREEMTKNQVSLTCLVKGFYPSDIAVEWESNGQPENNYKTTPPVLDSDGSFFLYSKLTVDKSRWQQGNVFSCSVMHEALHNHYTQKSLSLSPGK

SEQ ID NO: 31 - protein, 220 aa, Artificial Sequence
  hu2E5VL0CL
DIVMTQSPDSLAVSLGERATINCKSSQSLLYSRNQKNYLAWYQQKPGQPPKLLIYWASTRESGVPDRFSGSGSGTDFTLTISSLQAEDVAVYYCQQYYRYPLTFGGGTKVEIKRTVAAPSVFIFPPSDEQLKSGTASVVCLLNNFYPREAKVQWKVDNALQSGNSQESVTEQDSKDSTYSLSSTLTLSKADYEKHKVYACEVTHQGLSSPVTKSFNRGEC

SEQ ID NO: 32 - protein, 25 aa, Artificial Sequence
  m2E5 H-FR1; hu2E5 H-FR1
  misc_feature (3)..(3): Xaa = Lys or Gln
  misc_feature (4)..(4): Xaa = Leu or Val
  misc_feature (5)..(5): Xaa = Glu or Val
  misc_feature (11)..(11): Xaa = Leu or Ser
  misc_feature (18)..(18): Xaa = Leu or Met
  misc_feature (23)..(23): Xaa = Ala or Val
EVXXXESGGGXVQPGGSXKLSCXAS

SEQ ID NO: 33 - protein, 17 aa, Artificial Sequence
  m2E5 H-FR2; hu2E5 H-FR2
  misc_feature (7)..(7): Xaa = Ala or Ser
  misc_feature (8)..(8): Xaa = Pro or Ser
  misc_feature (9)..(9): Xaa = Glu or Gly
  misc_feature (16)..(16): Xaa = Ala or Gly
MNWVRQXXXKGLEWVXE

SEQ ID NO: 34 - protein, 38 aa, Artificial Sequence
  m2E5 H-FR3; hu2E5 H-FR3
  misc_feature (19)..(19): Xaa = Asn or Ser
  misc_feature (20)..(20): Xaa = Ser or Thr
  misc_feature (27)..(27): Xaa = Asn or Ser
  misc_feature (29)..(29): Xaa = Lys or Arg
  misc_feature (34)..(34): Xaa = Ala or Gly
  misc_feature (35)..(35): Xaa = Ile or Val
RYAESVKGRFTISRDDSKXXVYLQMNXLXTEDTXXYYC

SEQ ID NO: 35 - protein, 11 aa, Artificial Sequence
  m2E5 H-FR4; hu2E5 H-FR4
  misc_feature (7)..(7): Xaa = Leu or Val
WGQGTTXTVSS

SEQ ID NO: 36 - protein, 26 aa, Artificial Sequence
  m2E5 L-FR1; hu2E5 L-FR1
  misc_feature (5)..(5): Xaa = Ser or Thr
  misc_feature (9)..(9): Xaa = Asp or Ser
  misc_feature (12)..(12): Xaa = Ala or Gly
  misc_feature (15)..(15): Xaa = Leu or Val
  misc_feature (18)..(18): Xaa = Lys or Arg
  misc_feature (19)..(19): Xaa = Ala or Ile
  misc_feature (21)..(21): Xaa = Ile or Met
  misc_feature (22)..(22): Xaa = Asn or Ser
DIVMXQSPXSLXVSXGEXXTXXCKSS

SEQ ID NO: 37 - protein, 17 aa, Artificial Sequence
  m2E5 L-FR2; hu2E5 L-FR2
  misc_feature (11)..(11): Xaa = Pro or Ser
LAWYQQKPGQXPKLLIY

SEQ ID NO: 38 - protein, 37 aa, Artificial Sequence
  hu2E5 L-FR3; m2E5 L-FR3
  misc_feature (12)..(12): Xaa = Ser or Thr
  misc_feature (27)..(27): Xaa = Leu or Val
  misc_feature (28)..(28): Xaa = Lys or Gln
  misc_feature (32)..(32): Xaa = Leu or Val
STRESGVPDRFXGSGSGTDFTLTISSXXAEDXAVYYC

SEQ ID NO: 39 - protein, 124 aa, Artificial Sequence
  m2E5 VH; hu2E5 VH3
  misc_feature (3)..(3): Xaa = Lys or Gln
  misc_feature (4)..(4): Xaa = Leu or Val
  misc_feature (5)..(5): Xaa = Glu or Val
  misc_feature (11)..(11): Xaa = Leu or Ser
  misc_feature (18)..(18): Xaa = Leu or Met
  misc_feature (23)..(23): Xaa = Ala or Val
  misc_feature (40)..(40): Xaa = Ala or Ser
  misc_feature (41)..(41): Xaa = Pro or Ser
  misc_feature (42)..(42): Xaa = Glu or Gly
  misc_feature (49)..(49): Xaa = Ala or Gly
  misc_feature (79)..(79): Xaa = Asn or Ser
  misc_feature (80)..(80): Xaa = Ser or Thr
  misc_feature (87)..(87): Xaa = Asn or Ser
  misc_feature (89)..(89): Xaa = Lys or Arg
  misc_feature (94)..(94): Xaa = Ala or Gly
  misc_feature (95)..(95): Xaa = Ile or Val
  misc_feature (120)..(120): Xaa = Leu or Val
EVXXXESGGGXVQPGGSXKLSCXASGYTFGDNWMNWVRQXXXKGLEWVXEIRLKSNNYATRYAESVKGRFTISRDDSKXXVYLQMNXLXTEDTXXYYCTRTQFITSVVAPFDFWGQGTTXTVSS

SEQ ID NO: 40 - protein, 113 aa, Artificial Sequence
  m2E5 VL; hu2E5VL0
  misc_feature (5)..(5): Xaa = Ser or Thr
  misc_feature (9)..(9): Xaa = Asp or Ser
  misc_feature (12)..(12): Xaa = Ala or Gly
  misc_feature (15)..(15): Xaa = Leu or Val
  misc_feature (18)..(18): Xaa = Lys or Arg
  misc_feature (19)..(19): Xaa = Ala or Ile
  misc_feature (21)..(21): Xaa = Ile or Met
  misc_feature (22)..(22): Xaa = Asn or Ser
  misc_feature (49)..(49): Xaa = Pro or Ser
  misc_feature (69)..(69): Xaa = Ser or Thr
  misc_feature (84)..(84): Xaa = Leu or Val
  misc_feature (85)..(85): Xaa = Lys or Gln
  misc_feature (89)..(89): Xaa = Leu or Val
DIVMXQSPXSLXVSXGEXXTXXCKSSQSLLYSRNQKNYLAWYQQKPGQXPKLLIYWASTRESGVPDRFXGSGSGTDFTLTISSXXAEDXAVYYCQQYYRYPLTFGGGTKVEIK

SEQ ID NO: 41 - protein, 5 aa, Artificial Sequence
  HCDR1 (Kabat)
DNWMN

SEQ ID NO: 42 - protein, 19 aa, Artificial Sequence
  HCDR2 (Kabat)
EIRLKSNNYATRYAESVKG

SEQ ID NO: 43 - protein, 6 aa, Artificial Sequence
  HCDR3 (Kabat)
TQFITS

SEQ ID NO: 44 - protein, 17 aa, Artificial Sequence
  LCDR1 (Kabat)
KSSQSLLYSRNQKNYLA

SEQ ID NO: 45 - protein, 7 aa, Artificial Sequence
  LCDR2 (Kabat)
WASTRES

SEQ ID NO: 46 - protein, 10 aa, Artificial Sequence
  HCDR1 (combined)
GYTFGDNWMN